European Patent Application EP 4 194 544 A1, published June 14, 2023. Title: N-ACETYLGLUCOSAMINE-PRODUCING BACTERIAL STRAIN AS WELL AS METHOD OF CONSTRUCTION AND USE THEREOF. Applicant: Shanghai Jiao Tong University Anhui Yinchuang Biotechnology Co., Ltd. The sequence listing filed with the application follows.

SEQUENCE LISTING (34 sequences)

SEQ ID NO: 1 - DNA, 480 bp, Artificial Sequence
atgagcctgccggacggcttttatatccgccgcatggaagaaggcgacctggaacaggtcacggaaacgctgaaagtcctgacgacggtcggcacgatcacgccggaaagctttagcaaactgatcaaatattggaacgaagcgacggtctggaacgacaacgaagacaaaaaaatcatgcagtataacccgatggtcatcgtcgacaaacgcacggaaacggtcgcggcgacgggcaacatcatcatcgaacgcaaaatcatccatgaactgggcctgtgcggccatatcgaagacatcgcggtcaacagcaaatatcagggccagggcctgggcaaactgctgatcgaccagctcgtcactatcggcttcgactacggctgctataaaatcatcctggactgcgacgaaaagaatgtcaaattctacgaaaaatgcggctttagcaacgcgggcgtcgaaatgcagatccgcaaataa

SEQ ID NO: 2 - DNA, 1803 bp, Artificial Sequence
atgtgtggtattgtaggttatattggccagcttgatgcaaaggaaattttacttaaaggtttggagaagctggagtatcgcggctacgattcagctggaatcgctgtagcgaacgaagacggcgtacacgtgtttaaagaaaaaggacggatcgccgatcttcgcgcagccgttgatgcaaacgtgaagtcacaagcgggaatcggacacacgcgctgggcgactcacggagaaccgagccgtctaaacgctcatccgcatcaaagcgcatcaggccgttttacacttgttcataacggcgtcatcgaaaactatgttcaactgacgcgcgaatatttacacgatgtaacccttaaaagcgatacggatacagaggttgtcgttcaagtgatcgagcaattcgtcaataacggccttgacacagaagaagcgttccgccaaacgctcatgctgctcaaaggctcttatgcgattgcattattcgatcatgaaaacaaagaaacaatctatgttgcgaaaaataaaagcccgcttcttgtcggccttggagacaatttcaatgttgtcgcgtctgatgcgatggcgatgcttcaagtgacaaacgaatacgtggagcttatggataaagaaatggtgattgtcacagacaaaaaagtcgtgatcaaaaacctcgacggagaattgatgtcacgtgcctcatatattgcagagcttgatgcgagcgatatcgaaaaaggcacataccctcactacatgttaaaagaaatcgatgaacagccgcttgtcatgcggaaaatcattcagacgtaccaagatgaaaacggcaagctctccattcctggagacatttcaaacgctgttgctgaagccgaccgcgtctatatcattgcctgcggaactagctaccatgcaggtcttgtcggcaagcaatttattgaaacatgggcgaaagttccggctgaagtccatgtcgcaagcgaattctcttacaatatgccattgctttctgagaagccgctgtttatctttatttctcaaagcggagaaacggctgacagccgcgcggttctcgtacaggtgaaaaagctcggacacaaagcgctgacattgaccaacgtaccgggatccacgctttcccgtgaagcggactatacgcttttactgaatgccggccctgaaatcgcggtagcgtcaacaaaagcatatacggcgcaaatcgccgttctcgcaattttggcagccgtgactgcggaaagccgcggcaaagaactcggctttgatcttgtcaaagagctcggcattatcggaaacgcgatggaagccctttgcgaccaaaaagacgaaatggaaatgatcgcccgtgaatacttgaccgtaacacgcaatgcatttttcatcggccgcggcctcgactatttcgtctgcctcgaaggatccctgaagctgaaagagatttcttacattcaagctgaaggcttcgccggcggcgaattgaagcacggtacgatcgcattgatcgaagacggcacaccggtcatcgcccttgcgacacaggagcacgtcaacttaagcatccgcggaaacgtcaaagaagtgacagcccgcggcgccaacccttgcgtgatctccctgaaaggcctggaagaagcagacgaccgcttcgtcctgcctgaagtgcatccggagctcgcaccgctcgtctccgtcatcccgctgcagctgatcgcatactacgcagcgctgcaccgcggctgtgacgttgataagccacggaacctggcgaagagtgtgacggtggagtag

SEQ ID NO: 3 - DNA, 300 bp, Artificial Sequence
aaggtgacgcctatttcactttctagctgtttaatctgctggctgagcggaggctgagtcatgttcagccgaagagctgcttttccgaaatgcagttcttcggcaacaaccataaaataacgaagatggcgcagctccattaatcactcattcctttctgaatgcgatttcagtcgttttacatattaattgtaagacaaagaagtattggaaaacaatttccacaagatgtatatttaataatacaataattttattaaaaattcattgtaaatgaatgaaaatggaggagtgagggct

SEQ ID NO: 4 - DNA, 441 bp, Artificial Sequence
tgtcgacgtgcatgcaggccggggcatatgggaaacagcgcggacggagcggaatttccaatttcatgccgcagccgcctgcgctgttctcatttgcggcttccttgtagagctcagcattattgagtggatgattatattccttttgataggtggtatgttttcgcttgaacttttaaatacagccattgaacatacggttgatttaataactgacaaacatcaccctcttgctaaagcggccaaggacgctgccgccggggctgtttgcgtttttaccgtgatttcgtgtatcattggtttacttatttttttgccaaagctgtaatggctgaaaattcttacatttattttacatttttagaaatgggcgtgaaaaaaagcgcgcgattatgtaaaatataaagtgatagcggtaccattataggaggagtgagggct

SEQ ID NO: 5 - DNA, 140 bp, Artificial Sequence
catgatgtgggcgttttttttatacaaaaaaacgcactgatttacaaaaccttaacattcggttcaaaccctttttacatagaacctttactctatacgtgtaggacaaattacacattatacgcggaggagtgagggct

SEQ ID NO: 6 - DNA, 224 bp, Artificial Sequence
cagcataatgaacatttactcatgtctattttcgttcttttctgtatgaaaatagttatttcgagtctctacggaaatagcgagagatgatatacctaaatagagataaaatcatctcaaaaaaatgggtctactaaaatattattccatctattacaataaattcacagaatagtcttttaagtaagtctactctgaatttttttaaaggaggagtgagggct

SEQ ID NO: 7 - DNA, 39 bp, Artificial Sequence
ggtacccgggagctcatgaatgaggaggatcacacagtc

SEQ ID NO: 8 - DNA, 40 bp, Artificial Sequence
gaaggggcttatcttagttaaaacccctttcgatgatatt

SEQ ID NO: 9 - DNA, 38 bp, Artificial Sequence
aaaggggttttaactaagataagccccttctgaggaag

SEQ ID NO: 10 - DNA, 37 bp, Artificial Sequence
aagcaacttcagttttccggcattctccttatgtcaa

SEQ ID NO: 11 - DNA, 36 bp, Artificial Sequence
ggtacccgggagctctagggtaaaaccgtatgccgc

SEQ ID NO: 12 - DNA, 37 bp, Artificial Sequence; identical to SEQ ID NO: 10

SEQ ID NO: 13 - DNA, 40 bp, Artificial Sequence
aaggagaatgccggaaaactgaagttgcttttgaggaatc

SEQ ID NO: 14 - DNA, 36 bp, Artificial Sequence
gcgtcgggcgatatcggaaatttctctgccagctgc

SEQ ID NO: 15 - DNA, 37 bp, Artificial Sequence
ggtacccgggagctcggtcaagagggagggttcactt

SEQ ID NO: 16 - DNA, 40 bp, Artificial Sequence
tgtcagtcattcaatgtttttctcctttccacaaaataaa

SEQ ID NO: 17 - DNA, 40 bp, Artificial Sequence
ggaaaggagaaaaacattgaatgactgacaaaatcggtta

SEQ ID NO: 18 - DNA, 34 bp, Artificial Sequence
gcgtcgggcgatatctcatatcggggatcggctt

SEQ ID NO: 19 - DNA, 31 bp, Artificial Sequence
ggtacccgggagctcccgcacggtcagctta

SEQ ID NO: 20 - DNA, 40 bp, Artificial Sequence
gggaatcttttttgatacaactctagttgtctagaccaat

SEQ ID NO: 21 - DNA, 35 bp, Artificial Sequence
acaactagagttgtatcaaaaaagattcccacatt

SEQ ID NO: 22 - DNA, 36 bp, Artificial Sequence
gcgtcgggcgatatccctcttcatatcaatgacgaa

SEQ ID NO: 23 - DNA, 40 bp, Artificial Sequence
tatcgataagcttgatatcgaaggtgacgcctatttcact

SEQ ID NO: 24 - DNA, 33 bp, Artificial Sequence
gtccggcaggctcatagccctcactcctccatt

SEQ ID NO: 25 - DNA, 37 bp, Artificial Sequence
tatcgataagcttgatatcgtgtcgacgtgcatgcag

SEQ ID NO: 26 - DNA, 36 bp, Artificial Sequence
gtccggcaggctcatagccctcactcctcctataat

SEQ ID NO: 27 - DNA, 38 bp, Artificial Sequence
tatcgataagcttgatatcgcatgatgtgggcgttttt

SEQ ID NO: 28 - DNA, 33 bp, Artificial Sequence; identical to SEQ ID NO: 24

SEQ ID NO: 29 - DNA, 44 bp, Artificial Sequence
tatcgataagcttgatatcgcagcataatgaacatttactcatg

SEQ ID NO: 30 - DNA, 33 bp, Artificial Sequence; identical to SEQ ID NO: 24

SEQ ID NO: 31 - DNA, 31 bp, Artificial Sequence
ggaggagtgagggctatgagcctgccggacg

SEQ ID NO: 32 - DNA, 33 bp, Artificial Sequence
tacaataccacacattttgcggatctgcatttc

SEQ ID NO: 33 - DNA, 40 bp, Artificial Sequence
atgcagatccgcaaaatgtgtggtattgtaggttatattg

SEQ ID NO: 34 - DNA, 41 bp, Artificial Sequence
cggccgctctagaactagtgctactccaccgtcacactctt